European Patent Specification EP 3 603 659 B1, published October 8, 2025. Title: Pharmaceutical compositions for preventing and treating of inflammatory respiratory diseases comprising fusion protein of cell penetrating peptide and ctCTLA4 peptide. Applicant: IUCF-HYU(Industry-University Cooperation Foundation Hanyang University). The sequence listing filed with the application follows.

SEQUENCE LISTING (7 sequences)

SEQ ID NO: 1 - protein, 24 aa, Artificial Sequence
  dNP2 peptide
KIKKVKKKGRKGSKIKKVKKKGRK

SEQ ID NO: 2 - protein, 36 aa, Artificial Sequence
  ctCTLA-4 peptide
KMLKKRSPLTTGVYVKMPPTEPECEKQFQPYFIPIN

SEQ ID NO: 3 - protein, 11 aa, Artificial Sequence
  Hph-1 peptide
YARVRRRGPRR

SEQ ID NO: 4 - DNA, 67 bp, Artificial Sequence
  dNP2-ctCTLA-4 forward primer
aagattaagaaagtcaagaagaaaggaagaaaggaattctacccatacgatgttccagattacgcta

SEQ ID NO: 5 - DNA, 67 bp, Artificial Sequence
  dNP2-ctCTLA-4 forward primer
gctagcaagattaagaaagtcaagaagaaaggaagaaagggatccaagattaagaaagtcaagaaga

SEQ ID NO: 6 - DNA, 61 bp, Artificial Sequence
  dNP2-EGFP forward primer
aagattaagaaagtcaagaagaaaggaagaaaggtgagcaagggcgaggagctgttcaccg

SEQ ID NO: 7 - DNA, 67 bp, Artificial Sequence; identical to SEQ ID NO: 5
  dNP2-EGFP forward primer